European Patent Application EP 4 759 829 A1, published June 17, 2026. Title: 新規なＨＶＥＭ結合タンパク質およびそれを含む医薬組成物. Applicant: 国立大学法人　東京大学. Application JP. The sequence listing filed with the application follows.

SEQUENCE LISTING (35 sequences)

SEQ ID NO: 1 - protein, 10 aa, Vicugna pacos
GSIGSIHRWD

SEQ ID NO: 2 - protein, 9 aa, Vicugna pacos
TLNSEGGPT

SEQ ID NO: 3 - protein, 7 aa, Vicugna pacos
RTVPFEY

SEQ ID NO: 4 - protein, 25 aa, Vicugna pacos
QVQLVESGGGSVQPGGSLRLSCAAS

SEQ ID NO: 5 - protein, 25 aa, synthetic construct [sequence omitted]

SEQ ID NO: 6 - protein, 14 aa, Vicugna pacos
WYRLCPGKQREWVA

SEQ ID NO: 7 - protein, 14 aa, synthetic construct
WYRLSPGKQREWVA

SEQ ID NO: 8 - protein, 14 aa, synthetic construct
WYRQAPGKQREWVA

SEQ ID NO: 9 - protein, 39 aa, Vicugna pacos
YADSVEGRFTISRDNAKNMVYLQMNSLKPEDTAVYRCSA

SEQ ID NO: 10 - protein, 39 aa, synthetic construct
YADSVEGRFTISRDNSKNMVYLQMNSLRPEDTAVYRCSA

SEQ ID NO: 11 - protein, 39 aa, synthetic construct
YADSVEGRFTISRDNSKNTLYLQMNSLRPEDTAVYRCAA

SEQ ID NO: 12 - protein, 11 aa, Vicugna pacos
WGRGTQVTVSS

SEQ ID NO: 13 - protein, 11 aa, synthetic construct
WGQGTLVTVSS

SEQ ID NO: 14 - protein, 225 aa, Homo sapiens
GPPCPSCPAPEFLGGPSVFLFPPKPKDTLMISRTPEVTCVVVDVSQEDPEVQFNWYVDGVEVHNAKTKPREEQFNSTYRVVSVLTVLHQDWLNGKEYKCKVSNKGLPSSIEKTISKAKGQPREPQVYTLPPSQEEMTKNQVSLTCLVKGFYPSDIAVEWESNGQPENNYKTTPPVLDSDGSFFLYSRLTVDKSRWQEGNVFSCSVMHEALHNHYTQKSLSLSLGK

SEQ ID NO: 15 - protein, 229 aa, synthetic construct
ESKYGPPCPPCPAPEFLGGPSVFLFPPKPKDTLMISRTPEVTCVVVDVSQEDPEVQFNWYVDGVEVHNAKTKPREEQFNSTYRVVSVLTVLHQDWLNGKEYKCKVSNKGLPSSIEKTISKAKGQPREPQVYTLPPSQEEMTKNQVSLTCLVKGFYPSDIAVEWESNGQPENNYKTTPPVLDSDGSFFLYSRLTVDKSRWQEGNVFSCSVMHEALHNHYTQKSLSLSLGK

SEQ ID NO: 16 - protein, 225 aa, synthetic construct
GPPCPPCPAPEFLGGPSVFLFPPKPKDTLMISRTPEVTCVVVDVSQEDPEVQFNWYVDGVEVHNAKTKPREEQFNSTYRVVSVLTVLHQDWLNGKEYKCKVSNKGLPSSIEKTISKAKGQPREPQVYTLPPSQEEMTKNQVSLTCLVKGFYPSDIAVEWESNGQPENNYKTTPPVLDSDGSFFLYSRLTVDKSRWQEGNVFSCSVMHEALHNHYTQKSLSLSLGK

SEQ ID NO: 17 - protein, 115 aa, Vicugna pacos
QVQLVESGGGSVQPGGSLRLSCAASGSIGSIHRWDWYRLCPGKQREWVATLNSEGGPTYADSVEGRFTISRDNAKNMVYLQMNSLKPEDTAVYRCSARTVPFEYWGRGTQVTVSS

SEQ ID NO: 18 - protein, 115 aa, synthetic construct
EVQLVESGGGLVQPGGSLRLSCAASGSIGSIHRWDWYRLCPGKQREWVATLNSEGGPTYADSVEGRFTISRDNSKNMVYLQMNSLRPEDTAVYRCSARTVPFEYWGQGTLVTVSS

SEQ ID NO: 19 - protein, 115 aa, synthetic construct
EVQLVESGGGLVQPGGSLRLSCAASGSIGSIHRWDWYRLSPGKQREWVATLNSEGGPTYADSVEGRFTISRDNSKNMVYLQMNSLRPEDTAVYRCSARTVPFEYWGQGTLVTVSS

SEQ ID NO: 20 - protein, 115 aa, synthetic construct
EVQLVESGGGLVQPGGSLRLSCAASGSIGSIHRWDWYRQAPGKQREWVATLNSEGGPTYADSVEGRFTISRDNSKNTLYLQMNSLRPEDTAVYRCAARTVPFEYWGQGTLVTVSS

SEQ ID NO: 21 - protein, 340 aa, synthetic construct
QVQLVESGGGSVQPGGSLRLSCAASGSIGSIHRWDWYRLCPGKQREWVATLNSEGGPTYADSVEGRFTISRDNAKNMVYLQMNSLKPEDTAVYRCSARTVPFEYWGRGTQVTVSSGPPCPSCPAPEFLGGPSVFLFPPKPKDTLMISRTPEVTCVVVDVSQEDPEVQFNWYVDGVEVHNAKTKPREEQFNSTYRVVSVLTVLHQDWLNGKEYKCKVSNKGLPSSIEKTISKAKGQPREPQVYTLPPSQEEMTKNQVSLTCLVKGFYPSDIAVEWESNGQPENNYKTTPPVLDSDGSFFLYSRLTVDKSRWQEGNVFSCSVMHEALHNHYTQKSLSLSLGK

SEQ ID NO: 22 - protein, 344 aa, synthetic construct
QVQLVESGGGSVQPGGSLRLSCAASGSIGSIHRWDWYRLCPGKQREWVATLNSEGGPTYADSVEGRFTISRDNAKNMVYLQMNSLKPEDTAVYRCSARTVPFEYWGRGTQVTVSSESKYGPPCPPCPAPEFLGGPSVFLFPPKPKDTLMISRTPEVTCVVVDVSQEDPEVQFNWYVDGVEVHNAKTKPREEQFNSTYRVVSVLTVLHQDWLNGKEYKCKVSNKGLPSSIEKTISKAKGQPREPQVYTLPPSQEEMTKNQVSLTCLVKGFYPSDIAVEWESNGQPENNYKTTPPVLDSDGSFFLYSRLTVDKSRWQEGNVFSCSVMHEALHNHYTQKSLSLSLGK

SEQ ID NO: 23 - protein, 340 aa, synthetic construct
EVQLVESGGGLVQPGGSLRLSCAASGSIGSIHRWDWYRLCPGKQREWVATLNSEGGPTYADSVEGRFTISRDNSKNMVYLQMNSLRPEDTAVYRCSARTVPFEYWGQGTLVTVSSGPPCPSCPAPEFLGGPSVFLFPPKPKDTLMISRTPEVTCVVVDVSQEDPEVQFNWYVDGVEVHNAKTKPREEQFNSTYRVVSVLTVLHQDWLNGKEYKCKVSNKGLPSSIEKTISKAKGQPREPQVYTLPPSQEEMTKNQVSLTCLVKGFYPSDIAVEWESNGQPENNYKTTPPVLDSDGSFFLYSRLTVDKSRWQEGNVFSCSVMHEALHNHYTQKSLSLSLGK

SEQ ID NO: 24 - protein, 340 aa, synthetic construct
EVQLVESGGGLVQPGGSLRLSCAASGSIGSIHRWDWYRLSPGKQREWVATLNSEGGPTYADSVEGRFTISRDNSKNMVYLQMNSLRPEDTAVYRCSARTVPFEYWGQGTLVTVSSGPPCPSCPAPEFLGGPSVFLFPPKPKDTLMISRTPEVTCVVVDVSQEDPEVQFNWYVDGVEVHNAKTKPREEQFNSTYRVVSVLTVLHQDWLNGKEYKCKVSNKGLPSSIEKTISKAKGQPREPQVYTLPPSQEEMTKNQVSLTCLVKGFYPSDIAVEWESNGQPENNYKTTPPVLDSDGSFFLYSRLTVDKSRWQEGNVFSCSVMHEALHNHYTQKSLSLSLGK

SEQ ID NO: 25 - protein, 340 aa, synthetic construct
EVQLVESGGGLVQPGGSLRLSCAASGSIGSIHRWDWYRQAPGKQREWVATLNSEGGPTYADSVEGRFTISRDNSKNTLYLQMNSLRPEDTAVYRCAARTVPFEYWGQGTLVTVSSGPPCPPCPAPEFLGGPSVFLFPPKPKDTLMISRTPEVTCVVVDVSQEDPEVQFNWYVDGVEVHNAKTKPREEQFNSTYRVVSVLTVLHQDWLNGKEYKCKVSNKGLPSSIEKTISKAKGQPREPQVYTLPPSQEEMTKNQVSLTCLVKGFYPSDIAVEWESNGQPENNYKTTPPVLDSDGSFFLYSRLTVDKSRWQEGNVFSCSVMHEALHNHYTQKSLSLSLGK

SEQ ID NO: 26 - protein, 344 aa, synthetic construct
EVQLVESGGGLVQPGGSLRLSCAASGSIGSIHRWDWYRQAPGKQREWVATLNSEGGPTYADSVEGRFTISRDNSKNTLYLQMNSLRPEDTAVYRCAARTVPFEYWGQGTLVTVSSESKYGPPCPPCPAPEFLGGPSVFLFPPKPKDTLMISRTPEVTCVVVDVSQEDPEVQFNWYVDGVEVHNAKTKPREEQFNSTYRVVSVLTVLHQDWLNGKEYKCKVSNKGLPSSIEKTISKAKGQPREPQVYTLPPSQEEMTKNQVSLTCLVKGFYPSDIAVEWESNGQPENNYKTTPPVLDSDGSFFLYSRLTVDKSRWQEGNVFSCSVMHEALHNHYTQKSLSLSLGK

SEQ ID NO: 27 - protein, 6 aa, synthetic construct
HHHHHH

SEQ ID NO: 28 - protein, 121 aa, synthetic construct
EVQLVESGGGLVQPGGSLRLSCAASGSIGSIHRWDWYRLCPGKQREWVATLNSEGGPTYADSVEGRFTISRDNSKNMVYLQMNSLRPEDTAVYRCSARTVPFEYWGQGTLVTVSSHHHHHH

SEQ ID NO: 29 - DNA, 423 bp, synthetic construct
  source 1..423: mol_type = other DNA
atgggctggtcttgtattattctgtttctggtcgcaactgctacaggcgtgcattctcaggtgcagctcgtggagtctgggggaggctcggtgcagcctggggggtctttgagactctcctgtgcagcctctggaagcatcggcagtatccatcgttgggactggtaccgcctgtgtccagggaaacagcgcgagtgggtcgcaactcttaatagtgagggtggcccaacctatgcagactccgtagaaggccgattcaccatctccagagacaacgccaagaacatggtatatctgcaaatgaacagcctgaaacctgaggacacggccgtctataggtgtagcgcccgaaccgtcccgtttgaatactggggccgggggacccaggtcaccgtctcctcacatcatcatcatcatcactag

SEQ ID NO: 30 - DNA, 423 bp, synthetic construct
  source 1..423: mol_type = other DNA
atgggctggtcttgtattattctgtttctggtcgcaactgctacaggcgtgcattctcaggttcagctggttgaaagcggtggtgcactggttcagcctggtggtagcctgcgtctgagctgtgcagcaagcggttttccggttaatcgttatagcatgcgttggtatcgtcaggcaccgggtaaagaacgtgaatgggttgcaggtatgagcagtgccggtgatcgtagcagctatgaagatagcgttaaaggtcgttttaccatcagccgtgatgatgcacgtaataccgtttatctgcaaatgaatagcctgaaaccggaagataccgcagtgtattattgcaatgttaacgtgggctttgaatattggggtcagggcacccaggttaccgttagcagccatcatcatcatcatcactag

SEQ ID NO: 31 - RNA, 103 nt, synthetic construct
  source 1..103: mol_type = other RNA
gagcagttccggctcgcgcgcgttttagagctagaaatagcaagttaaaataaggctagtccgttatcaacttgaaaaagtggcaccgagtcggtgctttttt

SEQ ID NO: 32 - RNA, 103 nt, synthetic construct
  source 1..103: mol_type = other RNA
gccctccggacgtcaccacgggttttagagctagaaatagcaagttaaaataaggctagtccgttatcaacttgaaaaagtggcaccgagtcggtgctttttt

SEQ ID NO: 33 - RNA, 103 nt, synthetic construct
  source 1..103: mol_type = other RNA
ggtattactgatattggtggggttttagagctagaaatagcaagttaaaataaggctagtccgttatcaacttgaaaaagtggcaccgagtcggtgctttttt

SEQ ID NO: 34 - protein, 140 aa, synthetic construct
MGWSCIILFLVATATGVHSQVQLVESGGGSVQPGGSLRLSCAASGSIGSIHRWDWYRLCPGKQREWVATLNSEGGPTYADSVEGRFTISRDNAKNMVYLQMNSLKPEDTAVYRCSARTVPFEYWGRGTQVTVSSHHHHHH

SEQ ID NO: 35 - protein, 140 aa, synthetic construct
MGWSCIILFLVATATGVHSQVQLVESGGALVQPGGSLRLSCAASGFPVNRYSMRWYRQAPGKEREWVAGMSSAGDRSSYEDSVKGRFTISRDDARNTVYLQMNSLKPEDTAVYYCNVNVGFEYWGQGTQVTVSSHHHHHH